European Patent Application EP 4 176 899 A1, published May 10, 2023. Title: Porcine Circovirus Type 2 (PCV2) subunit vaccine. Applicant: BOEHRINGER INGELHEIM VETMEDICA INC. The sequence listing filed with the application follows.

SEQUENCE LISTING (3 sequences)

SEQ ID NO: 1 - protein, 234 aa, Porcine circovirus
MTYPRRRFRRRRHRPRSHLGQILRRRPWLVHPRHRYRWRRKNGIFNTRLSRTIGYTVKKTTVRTPSWNVDMMRFNINDFLPPGGGSNPLTVPFEYYRIRKVKVEFWPCSPITQGDRGVGSTAVILDDNFVTKANALTYDPYVNYSSRHTITQPFSYHSRYFTPKPVLDRTIDYFQPNNKRNQLWLRLQTTGNVDHVGLGTAFENSIYDQDYNIRITMYVQFREFNLKDPPLNPK

SEQ ID NO: 2 - protein, 233 aa, Porcine circovirus
MTYPRRRYRRRRHRPRSHLGQILRRRPWLVHPRHRYRWRRKNGIFNTRLSRTFGYTVKATTVTTPSWAVDMMRFNIDDFVPPGGGTNKISIPFEYYRIRKVKVEFWPCSPITQGDRGVGSTAVILDDNFVTKATALTYDPYVNYSSRHTIPQPFSYHSRYFTPKPVLDSTIDYFQPNNKRNQLWLRLQTSRNVDHVGLGTAFENSKYDQDYNIRVTMYVQFREFNLKDPPLEP

SEQ ID NO: 3 - DNA, 705 bp, Porcine circovirus
  source 1..705: mol_type = other DNA
atgacgtatccaaggaggcgtttccgcagacgaagacaccgcccccgcagccatcttggccagatcctccgccgccgcccctggctcgtccacccccgccaccgttaccgctggagaaggaaaaatggcatcttcaacacccgcctctcccgcaccatcggttatactgtcaagaaaaccacagtcagaacgccctcctggaatgtggacatgatgagatttaatattaatgattttcttcccccaggagggggctcaaaccccctcactgtgccctttgaatactacagaataaggaaggttaaggttgagttctggccctgctccccaatcacccagggtgacaggggagtgggctccactgctgttattctagatgataactttgtaacaaaggccaatgccctaacctatgacccctatgtaaactactcctcccgccataccataacccagcccttctcctaccactcccggtactttaccccgaaacctgtccttgataggacaatcgattacttccaacccaataacaaaagaaatcaactctggctgagactacaaactactggaaatgtagaccatgtaggcctcggcactgcgttcgaaaacagtatatacgaccaggactacaatatccgtataaccatgtatgtacaattcagagaatttaatcttaaagaccccccacttaaccctaagtga